European Patent Application EP 4 184 166 A1, published May 24, 2023. Title: Method for screening an inhibitor for metastasis of colorectal cancer. Applicant: IUCF-HYU (Industry-University Cooperation Foundation Hanyang University). The sequence listing filed with the application follows.

SEQUENCE LISTING (2 sequences)

SEQ ID NO: 1 - protein, 532 aa, ICAM-1
MAPSSPRPALPALLVLLGALFPGPGNAQTSVSPSKVILPRGGSVLVTCSTSCDQPKLLGIETPLPKKELLLPGNNRKVYELSNVQEDSQPMCYSNCPDGQSTAKTFLTVYWTPERVELAPLPSWQPVGKNLTLRCQVEGGAPRANLTVVLLRGEKELKREPAVGEPAEVTTTVLVRRDHHGANFSCRTELDLRPQGLELFENTSAPYQLQTFVLPATPPQLVSPRVLEVDTQGTVVCSLDGLFPVSEAQVHLALGDQRLNPTVTYGNDSFSAKASVSVTAEDEGTQRLTCAVILGNQSQETLQTVTIYSFPAPNVILTKPEVSEGTEVTVKCEAHPRAKVTLNGVPAQPLGPRAQLLLKATPEDNGRSFSCSATLEVAGQLIHKNQTRELRVLYGPRLDERDCPGNWTWPENSQQTPMCQAWGNPLPELKCLKDGTFPLPIGESVTVTRDLEGTYLCRARSTQGEVTRKVTVNVLSPRYEIVIITVVAAAVIMGTAGLSTYLYNRQRKIKKYRLQQAQKGTPMKPNTQATPP

SEQ ID NO: 2 - DNA, 1625 bp, ICAM-1
atggctcccagcagcccccggcccgcgctgcccgcactcctggtcctgctcggggctctgttcccaggacctggcaatgccgaattcccctcaaaagtcatcctgccccggggaggctccgtgctggtgacatgcagcacctcctgtgaccagcccaagttgttgggcatagagaccccgttgcctaaaaaggagttgctcctgcctgggaacaaccggaaggtgtatgaactgagcaatgtgcaagaagatagccaaccaatgtgctattcaaactgccctgatgggcagtcaacagctaaaaccttcctcaccgtgtactggactccagaacgggtggaactggcacccctcccctcttggcagccagtgggcaagaaccttaccctacgctgccaggtggagggtggggcaccccgggccaacctcaccgtggtgctgctccgtggggagaaggagctgaaacgggagccagctgtgggggagcccgctgaggtcacgaccacggtgctggtgaggagagatcaccatggagccaatttctcgtgccgcactgaactggacctgcggccccaagggctggagctgtttgagaacacctcggccccctaccagctccagacctttgtcctgccagcgactcccccacaacttgtcagcccccgggtcctagaggtggacacgcaggggaccgtggtctgttccctggacgggctgttcccagtctcggaggcccaggtccacctggcactgggggaccagaggttgaaccccacagtcacctatggcaacgactccttctcggccaaggcctcagtcagtgtgaccgcagaggacgagggcacccagcggctgacgtgtgcagtaatactggggaaccagagccaggagacactgcagacagtgaccatttacagttttccggcgcccaacgtgattctgacgaagccagaggtctcagaagggaccgaggtgacagtgaagtgtgaggcccaccctagagccaaggtgacgctgaatggggttccagcccagccactgggcccgagggcccagctcctgctgaaggccaccccagaggacaacgggcgcagcttctcctgctctgcaaccctggaggtggccggccagcttatacacaagaaccagacccgggagcttcgtgtcctgtatggcccccgactggacgagagggattgtccgggaaactggacgtggccagaaaattcccagcagactccaatgtgccaggcttgggggaacccattgcccgagctcaagtgtctaaaggatggcactttcccactgcccatcggggaatcagtgactgtcactcgagatcttgagggcacctacctctgtcgggccaggagcactcaaggggaggtcacccgcgaggtgaccgtgaatgtgctctccccccggtatgagattgtcatcatcactgtggtagcagccgcagtcataatgggcactgcaggcctcagcacgtacctctataaccgccagcggaagatcaagaaatacagactacaacaggcccaaaaagggacccccatgaaaccgaacacacaagccacgcctccctacccatacgatgttccagattacgcttgagcggccgc